European Patent Specification EP 3 310 928 B1, published December 25, 2024. Title: Nucleic Acid Amplification and Detection Assays. Applicant: Cambridge Molecular Diagnostics Ltd. The sequence listing filed with the application follows.

SEQUENCE LISTING (11 sequences)

SEQ ID NO: 1 - DNA, 49 bp, Artificial Sequence
  oligonucleotide to detect Ampicillin resistance gene bla
atctgtctatttcgttcatccatagttgcctgactccccgtcgtgtaga

SEQ ID NO: 2 - DNA, 49 bp, Artificial Sequence
  oligonucleotide to detect Kanamycin resistance gene kan
aaggacaattacaaacaggaatcgaatgcaaccggcgcaggaacactgc

SEQ ID NO: 3 - DNA, 49 bp, Artificial Sequence
  oligonucleotide to detect Chloramphenicol resistance gene cat
gcaagaatgtgaataaaggccggataaaacttgtgcttatttttcttta

SEQ ID NO: 4 - DNA, 23 bp, Artificial Sequence
  probe for Ampicillin
  misc_feature (23)..(23): Biotin label
tacgaacgatcaagacagatact

SEQ ID NO: 5 - DNA, 23 bp, Artificial Sequence
  probe for Kanamycin
  misc_feature (23)..(23): Biotin label
atctgtttgactttgtccttact

SEQ ID NO: 6 - DNA, 24 bp, Artificial Sequence
  probe for Chloramphenicol
  misc_feature (24)..(24): Biotin label
ctactttatattcattcttgcact

SEQ ID NO: 7 - DNA, 49 bp, Artificial Sequence; identical to SEQ ID NO: 1
  Thiol modified oligonucleotide to Ampicillin resistance gene bla
  misc_feature (1)..(1): Thiol modified

SEQ ID NO: 8 - DNA, 49 bp, Artificial Sequence; identical to SEQ ID NO: 2
  Thiol modified oligonucleotide to Kanamycin resistance gene kan
  misc_feature (1)..(1): Thiol modified

SEQ ID NO: 9 - DNA, 49 bp, Artificial Sequence; identical to SEQ ID NO: 3
  Thiol-modified oligonucleotide to Chloramphenicol resistance gene cat
  misc_feature (1)..(1): thiol modified

SEQ ID NO: 10 - protein, 10 aa, Artificial Sequence
  artificial
GSETVRFQSG

SEQ ID NO: 11 - protein, 10 aa, Artificial Sequence
  artificial
GSENLYFQSG